European Patent Specification EP 3 728 636 B1, published September 11, 2024. Title: PARTICLES ASSOCIATED WITH OLIGONUCLEOTIDES. Applicant: Cellular Research, Inc. Lam, Gretchen Yinbon Shum, Eleen. The sequence listing filed with the application follows.

SEQUENCE LISTING (5 sequences)

SEQ ID NO: 1 - DNA, 103 bp, Artificial Sequence
  Synthetic Oligonucleotide
  n (78)..(85): n = a, t, c, or g
  misc_feature (78)..(85): n is a, c, g, or t
tctctctctacacgacgctcttccgatctgatggatgactggcctgcgactacacgaggtagcggtgacttccaaggnnnnnnnntttttttttttttttttt

SEQ ID NO: 2 - DNA, 103 bp, Artificial Sequence
  Synthetic Oligonucleotide
  n (78)..(103): n = a, t, c, or g
  misc_feature (78)..(103): n is a, c, g, or t
tctctctctacacgacgctcttccgatctgatggatgactggcctgcgactacacgaggtagcggtgacttccaaggnnnnnnnnnnnnnnnnnnnnnnnnnn

SEQ ID NO: 3 - DNA, 121 bp, Artificial Sequence
  Synthetic Oligonucleotide
  n (75)..(85): n = a, t, c, or g
  misc_feature (78)..(85): n is a, c, g, or t
  n (104)..(121): n = a, t, c, or g
  misc_feature (104)..(121): n is a, c, g, or t
tctctctctacacgacgctcttccgatctgatggatgactggcctgcgactacacgaggtagcggtgacttccaaggnnnnnnnnttttttttttttttttttnnnnnnnnnnnnnnnnnn

SEQ ID NO: 4 - DNA, 13 bp, Artificial Sequence
  Synthetic Oligonucleotide
acaagtctgtctg

SEQ ID NO: 5 - DNA, 23 bp, Artificial Sequence
  Synthetic Oligonucleotide
cacacccaaaaggccacactggt